European Patent Application EP 4 497 836 A1, published January 29, 2025. Title: Method for constructing of gene network using a single cell transcriptome and discovery method of gene that is key to differentiation using the same. Applicant: Korea Advanced Institute of Science and Technology. Application KR. The sequence listing filed with the application follows.

SEQUENCE LISTING (37 sequences)

SEQ ID NO: 1 - RNA, 19 nt, synthetic construct
  source 1..19: mol_type = other RNA
ggtcgaacaggaaggttat

SEQ ID NO: 2 - RNA, 19 nt, synthetic construct
  source 1..19: mol_type = other RNA
ataaccttcctgttcgacc

SEQ ID NO: 3 - RNA, 25 nt, synthetic construct
  source 1..25: mol_type = other RNA
gaagatccagacaagagaatttcta

SEQ ID NO: 4 - RNA, 25 nt, synthetic construct
  source 1..25: mol_type = other RNA
tagaaattctcttgtctggatcttc

SEQ ID NO: 5 - RNA, 19 nt, synthetic construct
  source 1..19: mol_type = other RNA
tgaacggcatgaacacgta

SEQ ID NO: 6 - RNA, 19 nt, synthetic construct
  source 1..19: mol_type = other RNA
tacgtgttcatgccgttca

SEQ ID NO: 7 - DNA, 25 bp, synthetic construct
  source 1..25: mol_type = other DNA
tgatgacatcaagaaggtggtgaag

SEQ ID NO: 8 - DNA, 22 bp, synthetic construct
  source 1..22: mol_type = other DNA
tccttggaggccattgggccat

SEQ ID NO: 9 - DNA, 22 bp, synthetic construct
  source 1..22: mol_type = other DNA
gggaacagatgggcagaaatcg

SEQ ID NO: 10 - DNA, 22 bp, synthetic construct
  source 1..22: mol_type = other DNA
gctggcttttgaagactcctgc

SEQ ID NO: 11 - DNA, 21 bp, synthetic construct
  source 1..21: mol_type = other DNA
gaggtggctacacaatccsta

SEQ ID NO: 12 - DNA, 21 bp, synthetic construct
  source 1..21: mol_type = other DNA
acaccaggtgcatgaggtaac

SEQ ID NO: 13 - DNA, 22 bp, synthetic construct
  source 1..22: mol_type = other DNA
ggaacaccactacgccttcaac

SEQ ID NO: 14 - DNA, 22 bp, synthetic construct
  source 1..22: mol_type = other DNA
agtgcatcacctgttcgtaggc

SEQ ID NO: 15 - DNA, 19 bp, synthetic construct
  source 1..19: mol_type = other DNA
ttaaccactttgcagggga

SEQ ID NO: 16 - DNA, 20 bp, synthetic construct
  source 1..20: mol_type = other DNA
ttcttgtcggtgatggcgaa

SEQ ID NO: 17 - DNA, 20 bp, synthetic construct
  source 1..20: mol_type = other DNA
ggggaaagccaagtcctacc

SEQ ID NO: 18 - DNA, 20 bp, synthetic construct
  source 1..20: mol_type = other DNA
ccagcaatcaggtcgtgtct

SEQ ID NO: 19 - DNA, 20 bp, synthetic construct
  source 1..20: mol_type = other DNA
aaccttcaggagcgaagacg

SEQ ID NO: 20 - DNA, 20 bp, synthetic construct
  source 1..20: mol_type = other DNA
tcttcctcaccaagtgtcgc

SEQ ID NO: 21 - DNA, 20 bp, synthetic construct
  source 1..20: mol_type = other DNA
gcctatgccttggtggtact

SEQ ID NO: 22 - DNA, 20 bp, synthetic construct
  source 1..20: mol_type = other DNA
ccggccatgtagcttgtcat

SEQ ID NO: 23 - DNA, 21 bp, synthetic construct
  source 1..21: mol_type = other DNA
ctggaccttgggaagcttatt

SEQ ID NO: 24 - DNA, 20 bp, synthetic construct
  source 1..20: mol_type = other DNA
aaagagatccgagaccagga

SEQ ID NO: 25 - DNA, 21 bp, synthetic construct
  source 1..21: mol_type = other DNA
gaagcctcttgaccatagacc

SEQ ID NO: 26 - DNA, 23 bp, synthetic construct
  source 1..23: mol_type = other DNA
ggaggtctttcacggtgagattg

SEQ ID NO: 27 - DNA, 23 bp, synthetic construct
  source 1..23: mol_type = other DNA
caatctagcagacggaactgaac

SEQ ID NO: 28 - DNA, 23 bp, synthetic construct
  source 1..23: mol_type = other DNA
cggacagtattcagttcgtttcc

SEQ ID NO: 29 - DNA, 22 bp, synthetic construct
  source 1..22: mol_type = other DNA
agaagttggtgagcagcggctt

SEQ ID NO: 30 - DNA, 22 bp, synthetic construct
  source 1..22: mol_type = other DNA
cactgatggctccaacttgcga

SEQ ID NO: 31 - DNA, 21 bp, synthetic construct
  source 1..21: mol_type = other DNA
ggcagatttggcgaaaggaca

SEQ ID NO: 32 - DNA, 22 bp, synthetic construct
  source 1..22: mol_type = other DNA
ggtcctgaacacgatggttagc

SEQ ID NO: 33 - DNA, 22 bp, synthetic construct
  source 1..22: mol_type = other DNA
acttccgtctgggcattctgac

SEQ ID NO: 34 - DNA, 23 bp, synthetic construct
  source 1..23: mol_type = other DNA
gctgtaagcagagcatactcctc

SEQ ID NO: 35 - DNA, 58 bp, synthetic construct
  source 1..58: mol_type = other DNA
ccgggctatcaagaaccactggaatctcgagattccagtggttcttgatagctttttg

SEQ ID NO: 36 - DNA, 56 bp, synthetic construct
  source 1..56: mol_type = other DNA
ccggcagtctcaccaatttcagaaactcgagtttctgaaattggtgagactgtttt

SEQ ID NO: 37 - DNA, 58 bp, synthetic construct
  source 1..58: mol_type = other DNA
ccggggaacaccactacgccttcaactcgagttgaaggcgtagtggtgttcctttttg